European Patent Application EP 4 434 516 A2, published September 25, 2024. Title: MODULAR PLATFORM FOR TARGETED THERAPEUTICS. Applicant: Ramot at Tel-Aviv University Ltd. The sequence listing filed with the application follows.

SEQUENCE LISTING (18 sequences)

SEQ ID NO: 1 - RNA, 21 nt, synthetic construct
  modified_base 20..21: mod_base = OTHER; note = thymine
  misc_feature 1..21: note = CD45 sense SiRNA sequence
  modified_base 1: mod_base = cm
  modified_base 5: mod_base = cm
  modified_base 10..13: mod_base = um
  modified_base 18: mod_base = cm
  modified_base 20^21: mod_base = OTHER; note = phosphorothioate linkages
  source 1..21: mol_type = other RNA
  modified_base 2: mod_base = um
  modified_base 6: mod_base = um
ctggctgaatttcagagcatt

SEQ ID NO: 2 - RNA, 21 nt, synthetic construct
  modified_base 20..21: mod_base = OTHER; note = thymine
  misc_feature 1..21: note = CD45 anti-sense SiRNA sequence
  modified_base 13: mod_base = cm
  modified_base 16: mod_base = cm
  modified_base 20^21: mod_base = OTHER; note = phosphorothioate linkages
  source 1..21: mol_type = other RNA
tgctctgaaattcagccagtt

SEQ ID NO: 3 - RNA, 21 nt, synthetic construct
  modified_base 20..21: mod_base = OTHER; note = thymine
  misc_feature 1..21: note = Luc sense SiRNA sequence
  modified_base 1..3: mod_base = cm
  modified_base 5: mod_base = cm
  modified_base 7: mod_base = cm
  modified_base 12: mod_base = um
  modified_base 14: mod_base = cm
  modified_base 20..21: mod_base = OTHER; note = thymine
  modified_base 20^21: mod_base = OTHER; note = phosphorothioate linkages
  source 1..21: mol_type = other RNA
  modified_base 2..3: mod_base = um
  modified_base 8: mod_base = um
  modified_base 15..16: mod_base = um
  modified_base 17: mod_base = cm
cttacgctgagtacttcgatt

SEQ ID NO: 4 - RNA, 21 nt, synthetic construct
  modified_base 20..21: mod_base = OTHER; note = thymine
  misc_feature 1..21: note = Luc anti-sense SiRNA sequence
  modified_base 7: mod_base = um
  modified_base 11: mod_base = cm
  modified_base 16: mod_base = um
  modified_base 20^21: mod_base = OTHER; note = phosphorothioate linkages
  source 1..21: mol_type = other RNA
tcgaagtactcagcgtaagtt

SEQ ID NO: 5 - RNA, 25 nt, synthetic construct
  modified_base 25: mod_base = OTHER; note = thymine
  misc_feature 1..25: note = TNF alpha sense SiRNA sequence
  modified_base 1: mod_base = gm
  modified_base 4: mod_base = um
  modified_base 6: mod_base = OTHER; note = 2'-O-Methyl-Adenosine
  modified_base 12: mod_base = um
  modified_base 14: mod_base = cm
  modified_base 16: mod_base = cm
  modified_base 18: mod_base = um
  source 1..25: mol_type = other RNA
  modified_base 2: mod_base = um
gtctcagcctcttctcattcctgct

SEQ ID NO: 6 - RNA, 27 nt, synthetic construct
  misc_feature 1..27: note = TNF alpha anti-sense SiRNA sequence
  modified_base 3: mod_base = cm
  modified_base 9: mod_base = um
  modified_base 11: mod_base = OTHER; note = 2'-O-Methyl-Adenosine
  modified_base 13: mod_base = OTHER; note = 2'-O-Methyl-Adenosine
  modified_base 23: mod_base = gm
  modified_base 25: mod_base = cm
  source 1..27: mol_type = other RNA
  modified_base 26: mod_base = OTHER; note = 2'-O-Methyl-Adenosine
  modified_base 27: mod_base = um
agcaggaatgagaagaggctgagacat

SEQ ID NO: 7 - RNA, 25 nt, synthetic construct
  modified_base 25: mod_base = OTHER; note = thymine
  misc_feature 1..25: note = PLK1 sense SiRNA sequence
  modified_base 1: mod_base = gm
  modified_base 4: mod_base = um
  modified_base 6: mod_base = OTHER; note = 2'-O-Methyl-Adenosine
  modified_base 12: mod_base = OTHER; note = 2'-O-Methyl-Adenosine
  modified_base 14: mod_base = um
  modified_base 16: mod_base = cm
  modified_base 18: mod_base = um
  modified_base 24: mod_base = cm
  source 1..25: mol_type = other RNA
  modified_base 2: mod_base = cm
gcttaatgacgagttctttacttct

SEQ ID NO: 8 - RNA, 27 nt, synthetic construct
  misc_feature 1..27: note = PLK1 anti-sense SiRNA sequence
  modified_base 3: mod_base = OTHER; note = 2'-O-Methyl-Adenosine
  modified_base 9: mod_base = OTHER; note = 2'-O-Methyl-Adenosine
  modified_base 11: mod_base = OTHER; note = 2'-O-Methyl-Adenosine
  modified_base 13: mod_base = cm
  modified_base 23: mod_base = OTHER; note = 2'-O-Methyl-Adenosine
  modified_base 25: mod_base = cm
  source 1..27: mol_type = other RNA
  modified_base 26: mod_base = OTHER; note = 2'-O-Methyl-Adenosine
  modified_base 27: mod_base = gm
agaagtaaagaactcgtcattaagcag

SEQ ID NO: 9 - DNA, 20 bp, synthetic construct
  misc_feature 1..20: note = Single strand DNA oligonucleotide
  source 1..20: mol_type = other DNA
ttgtggaagggctcatgacc

SEQ ID NO: 10 - DNA, 20 bp, synthetic construct
  misc_feature 1..20: note = Single strand DNA oligonucleotide
  source 1..20: mol_type = other DNA
tcttctgggtggcagtgatg

SEQ ID NO: 11 - DNA, 21 bp, synthetic construct
  misc_feature 1..21: note = Single strand DNA oligonucleotide
  source 1..21: mol_type = other DNA
gcaccaccatcaaggactcaa

SEQ ID NO: 12 - DNA, 20 bp, synthetic construct
  misc_feature 1..20: note = Single strand DNA oligonucleotide
  source 1..20: mol_type = other DNA
tcgaggctccagtgaattcg

SEQ ID NO: 13 - protein, 6 aa, synthetic construct
  REGION 1..6: note = first six amino acid of NlpA can be used as an N terminal anchor
CDQSSS

SEQ ID NO: 14 - protein, 117 aa, synthetic construct
  REGION 1..117: note = VH domain of the antibody
EVQLLQSGPELVKPGASVKIPCKASGYTFTDYNMDWVKQSHEKSLEWIGYINPYSGDTIYNHKFKDKATLTVYKSSNIAYMELRSLTSEDTAVYYCARGGYDYGDHWGQGTTLTVSS

SEQ ID NO: 15 - protein, 107 aa, synthetic construct
  REGION 1..107: note = amino acid sequence of the VL domain (kappa) of the antibody
DIKMTQSPSSMYASLGERVTITCKASQDINSYLSWFQQKPGKSPKTLIYRANRLVDGVPSRFSGSGSGQDYSLTISSLEYEDMGIYYCLQDDEFPRTFGGGTKLEIK

SEQ ID NO: 16 - protein, 18 aa, synthetic construct
  REGION 1..18: note = linker sequence of the antibody
GSAGGGGSGGGGSGGGGS

SEQ ID NO: 17 - protein, 6 aa, synthetic construct
  REGION 1..6: note = short peptide
CDNSSS

SEQ ID NO: 18 - protein, 15 aa, synthetic construct
  REGION 1..15: note = Biotin lygase tag
LHHILDAQKMVWNHR